European Patent Application EP 4 621 052 A1, published September 24, 2025. Title: IMMUNE CELL TARGETING PROBE, CELL PRE-TARGETING RECOGNITION AND CELL BASED DRUG DELIVERY SYSTEM BASED ON PROBE, AND USE THEREOF. Applicant: GUANGDONG KEYANGLE LIFE TECHNOLOGY CO., LTD. Application EP. The sequence listing filed with the application follows.

SEQUENCE LISTING (32 sequences)

SEQ ID NO: 1 - protein, 23 aa, Gallus gallus
LQPDPGAVAAAAVLRAVLEGLQG

SEQ ID NO: 2 - protein, 26 aa, Rattus norvegicus
DQPDPGAVAAAAIFRAILEVLQTKAA

SEQ ID NO: 3 - protein, 26 aa, Canis lupus
DQPDPGAVAAAAILRTILEVLQSQGV

SEQ ID NO: 4 - protein, 26 aa, Sus scrofa
DQPDPGAVAAAAILRAILEVLQSQGA

SEQ ID NO: 5 - protein, 26 aa, Bos taurus
DQPDPGAVAAAAILRAILEVLQSQGA

SEQ ID NO: 6 - protein, 23 aa, Macaca mulatta
EQPDPGAVAAAAILRAILEVLQS

SEQ ID NO: 7 - protein, 27 aa, Mus musculus
LDQPDPGAVAAAAIFRAILEVLQTQGA

SEQ ID NO: 8 - protein, 8 aa, Homo sapiens
AILEVLQS

SEQ ID NO: 9 - protein, 10 aa, Homo sapiens
LRAILEVLQS

SEQ ID NO: 10 - protein, 11 aa, Homo sapiens
ILRAILEVLQS

SEQ ID NO: 11 - protein, 13 aa, Homo sapiens
AAILRAILEVLQS

SEQ ID NO: 12 - protein, 23 aa, Homo sapiens
EQPDPGAVAAAAILRAILEVLQS

SEQ ID NO: 13 - protein, 19 aa, Homo sapiens
PGAVAAAAILRAILEVLQS

SEQ ID NO: 14 - protein, 41 aa, Homo sapiens
KNMEAGAGRASYISSARLEQPDPGAVAAAAILRAILEVLQS

SEQ ID NO: 15 - protein, 8 aa, synthetic construct
AVLEVLQG

SEQ ID NO: 16 - protein, 11 aa, synthetic construct
VLRAVLEVLQG

SEQ ID NO: 17 - protein, 23 aa, synthetic construct
EQPDPSAVAAAAILRAILEVLQG

SEQ ID NO: 18 - protein, 23 aa, synthetic construct
LQPDPSAVAAAAVLRAVLEVLQG

SEQ ID NO: 19 - protein, 445 aa, synthetic construct
DVKIVESGGGLVKLGGSLKLSCAASGFTFSRNYMSWVRQTPEKRLELVAGINNNGGSTYYPDTVKGRFTISRDNAKNTLYLQMSSLRSEDTAIYYCAKRGFITTVGAMDYWGQGISVTVSSAKTTPPSVYPLAPGSAAQTNSMVTLGCLVKGYFPEPVTVTWNSGSLSSGVHTFPAVLQSDLYTLSSSVTVPSSTWPSETVTCNVAHPASSTKVDKKIVPRDCGCKPCICTVPEVSSVFIFPPKPKDVLTITLTPKVTCVVVDISKDDPEVQFSWFVDDVEVHTAQTQPREEQFNSTFRSVSELPIMHQDWLNGKEFKCRVNSAAFPAPIEKTISKTKGRPKAPQVYTIPPPKEQMAKDKVSLTCMITDFFPEDITVEWQWNGQPAENYKNTQPIMDTDGSYFVYSKLNVQKSNWEAGNTFTCSVLHEGLHNHHTEKSLSHSPGK

SEQ ID NO: 20 - DNA, 1338 bp, synthetic construct
  source 1..1338: mol_type = other DNA
gatgtgaagatagtggaaagtggtggtggattggtcaaacttggggggtccctgaaactcagctgcgctgccagcggcttcacatttagtagaaactacatgtcctgggtgaggcaaacgccagagaagcggctggagcttgtagctggcatcaacaacaatggaggcagcacctactatcctgacacagtcaaaggacgcttcaccatatccagagacaatgcaaagaataccctgtatctgcagatgtcatctttacgatcagaagatactgcaatctattactgtgccaagaggggttttattacaactgtgggggccatggactactggggccagggcatttctgttactgtgtcctccgccaagaccacaccaccttccgtctatcccttggcaccaggatcagccgcccaaactaacagtatggtgacactgggatgcctggttaagggctatttccctgagccagtgacagtgacttggaacagtggtagcctgagttcaggggtccacactttccccgctgtcttgcagagtgatctgtataccctcagctcctcagtgaccgttcctagcagtacgtggccttccgagactgtgacatgtaatgtagcccatcccgcttcatctaccaaggtggataagaagattgttccacgggactgcgggtgtaaaccgtgtatttgtactgtacccgaggtgagttccgttttcattttccctcccaagcccaaagatgttctcacaattactctgacaccaaaagttacatgcgtggtggtggacatcagcaaggacgatcctgaggtgcagttttcctggtttgttgatgacgtcgaagtccacactgcacagacccagccaagggaagaacagttcaatagtacattcagatccgtgtccgaattgccgattatgcatcaggactggctcaatggcaaagaatttaagtgtagagtgaactctgccgcctttcctgctcctatcgaaaagacaatcagcaagactaagggcagacctaaagccccccaagtgtatactattccaccccccaaagaacagatggccaaggacaaagtaagtttgacctgtatgatcactgacttcttcccagaagatatcactgtggaatggcagtggaacggacagcctgcggagaactataaaaatactcagcccattatggacacagacgggtcttacttcgtctacagtaaactgaatgttcagaaaagtaattgggaggccggcaatacattcacctgttcagtgctgcatgaggggcttcacaaccaccacactgagaaatcccttagccacagccctggcaagtaa

SEQ ID NO: 21 - protein, 214 aa, synthetic construct
DIQMTQTTFSLSASLGDRVTISCRASQDISNYLNWYQQIPDGTVKLLIYYTSRLHSGVPSRFSGSGSGTDYSLTISNLEQEDIATYFCQQVHTLPYTFGGGTKLEMKRADAAPTVSIFPPSSEQLTSGGASVVCFLNNFYPKDINVKWKIDGSERQNGVLNSWTDQDSKDSTYSMSSTLTLTKDEYERHNSYTCEATHKTSTSPIVKSFNRNEC

SEQ ID NO: 22 - DNA, 645 bp, synthetic construct
  source 1..645: mol_type = other DNA
gacattcagatgacccagacgaccttcagcctctctgcatcccttggagacagagtcaccatcagctgtcgggccagccaagatatatcaaattatctgaactggtaccagcagatcccagatggcactgtgaagctgcttatctactacacatcacgcctacattctggtgttccttccaggttttctgggagtggcagtgggacagactattccctcaccattagcaacctggagcaggaagatattgctacttacttctgccagcaagtgcacacactgccctatacttttggaggtggcaccaaattggagatgaaacgggccgatgctgctcctaccgtcagtatcttcccaccttcaagcgaacagcttaccagtggcggggcatctgtggtgtgcttcctgaataacttttacccaaaggatataaacgtgaagtggaagatcgacggcagcgagcggcaaaatggagtgttgaatagttggactgaccaggactctaaggactccacctactctatgtcatctacacttacactgacaaaggatgagtacgaacggcacaactcctatacatgcgaagctacccataagaccagtaccagccccattgtgaagtcattcaatagaaatgagtgctaa

SEQ ID NO: 23 - DNA, 52 bp, synthetic construct
  source 1..52: mol_type = other DNA
ggcctccggactctagaggatccgccaccatggagacagacacactcctgct

SEQ ID NO: 24 - DNA, 39 bp, synthetic construct
  source 1..39: mol_type = other DNA
ctcgagctaagcttcgaattcttacttgccagggctgtg

SEQ ID NO: 25 - DNA, 57 bp, synthetic construct
  source 1..57: mol_type = other DNA
cagaattcgaagcttagctcgagagccaccatggagacagacacactcctgctatgg

SEQ ID NO: 26 - DNA, 42 bp, synthetic construct
  source 1..42: mol_type = other DNA
cagaggttgattgtcgagatatcaaactcattactaaccggt

SEQ ID NO: 27 - protein, 19 aa, synthetic construct
KEQPDPGAVAAAAILRAIL

SEQ ID NO: 28 - protein, 22 aa, synthetic construct
KEQPDPGAVAAAAILRAILEVL

SEQ ID NO: 29 - protein, 24 aa, synthetic construct
KEQPDPGAVAAAAILRAILEVLQS

SEQ ID NO: 30 - protein, 29 aa, synthetic construct
KSSARLEQPDPGAVAAAAILRAILEVLQS

SEQ ID NO: 31 - protein, 23 aa, synthetic construct
EQPDPGAVAAAAILRAILEVLQS

SEQ ID NO: 32 - protein, 28 aa, synthetic construct
SSARLEQPDPGAVAAAAILRAILEVLQS